European Patent Specification EP 3 749 785 B1, published June 21, 2023. Title: SYSTEM AND PRODUCTS FOR IMPROVED QUANTIFICATION OF ADCC and ADCP ACTIVITY. Applicant: Euro Diagnostica AB. The sequence listing filed with the application follows.

SEQUENCE LISTING (1 sequence)

SEQ ID NO: 1 - DNA, 125 bp, Artificial
  Artifical
ggaagcgaaaatgaaattgactgggactttccggaggaaaaactgtttcatacagaaggcgtggatgtccatattaggatgagtcagtgacgtcagagcctgatttccccgaaatgatgagctag